European Patent Application EP 4 350 006 A1, published April 10, 2024. Title: NUCLEIC ACID COMBINATION FOR LIVER CANCER DIAGNOSIS OR AIDED DIAGNOSIS, TEST KIT, AND APPLICATION. Applicant: Wuhan Ammunition Life-tech Co.,Ltd. The sequence listing filed with the application follows.

SEQUENCE LISTING (58 sequences)

SEQ ID NO: 1 - DNA, 22 bp, Artificial Sequence
  Primer
tacgtacgggttcgtgttttga

SEQ ID NO: 2 - DNA, 22 bp, Artificial Sequence
  Primer
atcgacgatccaaatcctacaa

SEQ ID NO: 3 - DNA, 21 bp, Artificial Sequence
  Probe
tggaaggaggtttcggggagt

SEQ ID NO: 4 - DNA, 20 bp, Artificial Sequence
  Primer
atcgttcgggaagtgtttgc

SEQ ID NO: 5 - DNA, 20 bp, Artificial Sequence
  Primer
aactcgaacgaccgacgcta

SEQ ID NO: 6 - DNA, 21 bp, Artificial Sequence
  Probe
tcgtggggttagttttcgcgt

SEQ ID NO: 7 - DNA, 19 bp, Artificial Sequence
  Primer
ttattcgggtttcgtttcg

SEQ ID NO: 8 - DNA, 22 bp, Artificial Sequence
  Primer
actccctccaaataaacgacga

SEQ ID NO: 9 - DNA, 24 bp, Artificial Sequence
  Probe
tttacgtttttgcgagaagttcgg

SEQ ID NO: 10 - DNA, 19 bp, Artificial Sequence
  Primer
ttgtcggtgttcgttgggc

SEQ ID NO: 11 - DNA, 25 bp, Artificial Sequence
  Primer
atataaccgacgactctaatctcga

SEQ ID NO: 12 - DNA, 25 bp, Artificial Sequence
  Probe
tagtagtttttggagcgcggagtcg

SEQ ID NO: 13 - DNA, 24 bp, Artificial Sequence
  Primer
atagtcgagattagagtcgtcggt

SEQ ID NO: 14 - DNA, 19 bp, Artificial Sequence
  Primer
acaaaaactacgcgcgacg

SEQ ID NO: 15 - DNA, 25 bp, Artificial Sequence
  Probe
ttagtagttaatttcgcggcgcgtc

SEQ ID NO: 16 - DNA, 21 bp, Artificial Sequence
  Primer
tcggaaaggaaattggttacg

SEQ ID NO: 17 - DNA, 20 bp, Artificial Sequence
  Primer
tcattcccgaacaatttcgt

SEQ ID NO: 18 - DNA, 25 bp, Artificial Sequence
  Probe
ttagacgggcgttatttagtagcgt

SEQ ID NO: 19 - DNA, 25 bp, Artificial Sequence
  Primer
gagaaaataggaagtagaagttgcg

SEQ ID NO: 20 - DNA, 20 bp, Artificial Sequence
  Primer
acccgacgaaaacgtaccga

SEQ ID NO: 21 - DNA, 22 bp, Artificial Sequence
  Probe
ttcgtttttcgttcgggttgcg

SEQ ID NO: 22 - DNA, 21 bp, Artificial Sequence
  Primer
ttggtttcggttgtgagttgc

SEQ ID NO: 23 - DNA, 20 bp, Artificial Sequence
  Primer
ctacgaaaaacccgaaatcg

SEQ ID NO: 24 - DNA, 25 bp, Artificial Sequence
  Probe
tttaggggttgttgagcgtttagcg

SEQ ID NO: 25 - DNA, 23 bp, Artificial Sequence
  Primer
ttgtgtcgcgtttagttgttacg

SEQ ID NO: 26 - DNA, 20 bp, Artificial Sequence
  Primer
tacaaaacttaaaccgccga

SEQ ID NO: 27 - DNA, 25 bp, Artificial Sequence
  Probe
aattggttttacgatcgtcggcgta

SEQ ID NO: 28 - DNA, 23 bp, Artificial Sequence
  Primer
aaggtggttgggtggttgttttg

SEQ ID NO: 29 - DNA, 19 bp, Artificial Sequence
  Primer
aataacacccccaccctgc

SEQ ID NO: 30 - DNA, 19 bp, Artificial Sequence
  Probe
ggagtggtttttgggtttg

SEQ ID NO: 31 - DNA, 693 bp, Homo Sapiens  Homo sapiens)
cacgcacgggctcgtgctctgagttcctggaaggaggcctcggggagtgacgagaaaccaggggggtctgcaggacttggaccgccgaccgttcctcgctccccggggcgagcggtctggaccgcccgggaagtgcctgcgccggcggtcgtggggccagttcccgcgtggcagctgggcgcgacacaggcgcgccctcctcgtccctcccgggcagcgtcggccgcccgagcccggggagacccgccccgccccgcgccgtcacccgggccccgttccgcaggggtggctcgcggcgccccacgtccctgcgagaagcccgggatcgcttcgcggggcgcaccgacgagccgccgctcgcgagctcgccgcctacctggagggagctcaggcccgcgtcgaccgcgcgctgccggtgtccgctgggcgctcagcagcccctggagcgcggagccggcgtggagagcgcagctcacagccgagaccagagccgccggccacacccagtcccgcacctcccagcagccaactccgcggcgcgccggagccggggcggggacgtggctggaggcgcgaggcgcgaggcacgaggcgcgcgggcccggcggggacgtgccggggacgcgcagaccctcggagcgcgcgcagcccgggcggggggcgaagggagcgggcgccgcgcgcagcttctgc

SEQ ID NO: 32 - DNA, 766 bp, Homo Sapiens
ccggaaaggaaactggccacgccacttagacgggcgctacttagcagcgtgccccggcgccacaccaacaagaaaacgaaactgcccgggaatgaatgtttttcttctccttctggcaggaaacgagagagaaaataggaagcagaagctgcgcgcggcgcccgctcccttcgccccccgcccgggctgcgcgcgctccgagggtctgcgcgtccccggcacgtccccgccgggcccgcgcgcctcgtgcctcgcgcctcgcgcctccagccacgtccccgccccggctccggcgcgccgcggagttggctgctgggaggtgcgggactgggtgtggccggcggctctggtctcggctgtgagctgcgctctccacgccggctccgcgctccaggggctgctgagcgcccagcggacaccggcagcgcgcggtcgacgcgggcctgagctccctccaggtaggcggcgagctcgcgagcggcggctcgtcggtgcgccccgcgaagcgatcccgggcttctcgcagggacgtggggcgccgcgagccacccctgcggaacggggcccgggtgacggcgcggggcggggcgggtctccccgggctcgggcggccgacgctgcccgggagggacgaggagggcgcgcctgtgtcgcgcccagctgccacgcgggaactggccccacgaccgccggcgcaggcacttcccgggcggtccagaccgctcgccccggggagcgaggaacggtcggcggtccaagtcctgca

SEQ ID NO: 33 - DNA, 89 bp, Homo Sapiens
cacgcacgggctcgtgctctgagttcctggaaggaggcctcggggagtgacgagaaaccaggggggtctgcaggacttggaccgccgac

SEQ ID NO: 34 - DNA, 114 bp, Homo Sapiens
accgcccgggaagtgcctgcgccggcggtcgtggggccagttcccgcgtggcagctgggcgcgacacaggcgcgccctcctcgtccctcccgggcagcgtcggccgcccgagcc

SEQ ID NO: 35 - DNA, 126 bp, Homo Sapiens
tcacccgggccccgttccgcaggggtggctcgcggcgccccacgtccctgcgagaagcccgggatcgcttcgcggggcgcaccgacgagccgccgctcgcgagctcgccgcctacctggagggagc

SEQ ID NO: 36 - DNA, 94 bp, Homo Sapiens
ctgccggtgtccgctgggcgctcagcagcccctggagcgcggagccggcgtggagagcgcagctcacagccgagaccagagccgccggccacac

SEQ ID NO: 37 - DNA, 219 bp, Homo Sapiens
acagccgagaccagagccgccggccacacccagtcccgcacctcccagcagccaactccgcggcgcgccggagccggggcggggacgtggctggaggcgcgaggcgcgaggcacgaggcgcgcgggcccggcggggacgtgccggggacgcgcagaccctcggagcgcgcgcagcccgggcggggggcgaagggagcgggcgccgcgcgcagcttctgc

SEQ ID NO: 38 - DNA, 95 bp, Homo Sapiens
ccggaaaggaaactggccacgccacttagacgggcgctacttagcagcgtgccccggcgccacaccaacaagaaaacgaaactgcccgggaatga

SEQ ID NO: 39 - DNA, 107 bp, Homo Sapiens
gagaaaataggaagcagaagctgcgcgcggcgcccgctcccttcgccccccgcccgggctgcgcgcgctccgagggtctgcgcgtccccggcacgtccccgccgggc

SEQ ID NO: 40 - DNA, 180 bp, Homo Sapiens
ctggtctcggctgtgagctgcgctctccacgccggctccgcgctccaggggctgctgagcgcccagcggacaccggcagcgcgcggtcgacgcgggcctgagctccctccaggtaggcggcgagctcgcgagcggcggctcgtcggtgcgccccgcgaagcgatcccgggcttctcgcag

SEQ ID NO: 41 - DNA, 121 bp, Homo Sapiens
ctgtgtcgcgcccagctgccacgcgggaactggccccacgaccgccggcgcaggcacttcccgggcggtccagaccgctcgccccggggagcgaggaacggtcggcggtccaagtcctgca

SEQ ID NO: 42 - DNA, 25 bp, Artificial Sequence
  Probe
ctaggacgatttcggttgtattatt

SEQ ID NO: 43 - DNA, 25 bp, Artificial Sequence
  Primer
ctccctaacgacaaataaaacaaac

SEQ ID NO: 44 - DNA, 25 bp, Artificial Sequence
  Probe
ttgttggattggttcgttacgttgt

SEQ ID NO: 45 - DNA, 18 bp, Artificial Sequence
  Primer
gcgcgttgtttcgtttcg

SEQ ID NO: 46 - DNA, 20 bp, Artificial Sequence
  Primer
cgtcacctaccgcaaatacg

SEQ ID NO: 47 - DNA, 21 bp, Artificial Sequence
  Probe
ccacggacggcggataaggag

SEQ ID NO: 48 - DNA, 17 bp, Artificial Sequence
  Primer
gcgcgggaggattttcg

SEQ ID NO: 49 - DNA, 18 bp, Artificial Sequence
  Primer
ccgccaccataaacgacc

SEQ ID NO: 50 - DNA, 21 bp, Artificial Sequence
  Probe
ccacggacgcgaaatcgaaat

SEQ ID NO: 51 - DNA, 25 bp, Artificial Sequence
  Primer
gtacgtgacggtgttagttaatggt

SEQ ID NO: 52 - DNA, 19 bp, Artificial Sequence
  Primer
acgacgaaacgccgaaaat

SEQ ID NO: 53 - DNA, 25 bp, Artificial Sequence
  Probe
agtttgtcggttttcgtagtgatgg

SEQ ID NO: 54 - DNA, 22 bp, Artificial Sequence
  Primer
ttcgttggaagaagtttgtagg

SEQ ID NO: 55 - DNA, 25 bp, Artificial Sequence
  Primer
acgcttattcctacgatatcgtatc

SEQ ID NO: 56 - DNA, 24 bp, Artificial Sequence
  Probe
acgggaatttttttcgtcggtttc

SEQ ID NO: 57 - DNA, 858 bp, Homo Sapiens
cgccggaaaggaaactggccacgccacttagacgggcgctacttagcagcgtgccccggcgccacaccaacaagaaaacgaaactgcccgggaatgaatgtttttcttctccttctggcaggaaacgagagagaaaataggaagcagaagctgcgcgcggcgcccgctcccttcgccccccgcccgggctgcgcgcgctccgagggtctgcgcgtccccggcacgtccccgccgggcccgcgcgcctcgtgcctcgcgcctcgcgcctccagccacgtccccgccccggctccggcgcgccgcggagttggctgctgggaggtgcgggactgggtgtggccggcggctctggtctcggctgtgagctgcgctctccacgccggctccgcgctccaggggctgctgagcgcccagcggacaccggcagcgcgcggtcgacgcgggcctgagctccctccaggtaggcggcgagctcgcgagcggcggctcgtcggtgcgccccgcgaagcgatcccgggcttctcgcagggacgtggggcgccgcgagccacccctgcggaacggggcccgggtgacggcgcggggcggggcgggtctccccgggctcgggcggccgacgctgcccgggagggacgaggagggcgcgcctgtgtcgcgcccagctgccacgcgggaactggccccacgaccgccggcgcaggcacttcccgggcggtccagaccgctcgccccggggagcgaggaacggtcggcggtccaagtcctgcagacccccctggtttctcgtcactccccgaggcctccttccaggaactcagagcacgagcccgtgcgtgcccccaaaataacgggtattcg

SEQ ID NO: 58 - DNA, 560 bp, Homo Sapiens
cgcccggctcaaccccgacgtccgcgccccggccgcctgttggccatggcgggcctgggcctgggctccgccgttcccgtgtggctggccgaggacgacctcggctgcatcatctgccaggggctgctggactggcccgccacgctgccctgcggccacagcttctgccgccactgcctggaggccctgtggggcgcccgcgacgcccgccgctgggcctgccccacttgccgccagggcgccgcgcagcagccgcacctgcggaagaacacgctactgcaggacctggccgacaagtaccgccgcgccgcacgcgagatacaggcgggctccgaccctgcccactgcccctgcccgggctccagttccctctccagcgcggccgcgaggccccggcgccgcccggaactgcagcgggtagggaggccgggcccgcagctcccctggctcccccgggctgcccgccgcctgaccctttcccatgtggctcgaacccctttcctcagccgttctacttttacgttccttttctcagtctaaaagtcgagttccgctcttcg